European Patent Application EP 4 435 098 A1, published September 25, 2024. Title: CHIMERIC DNA POLYMERASE AND USE THEREOF. Applicant: BGI SHENZHEN. The sequence listing filed with the application follows.

SEQUENCE LISTING (34 sequences)

SEQ ID NO: 1 - protein, 778 aa, Artificial
  1
MASAILDTDYITENGKPVIRVFKKENGEFKIEYDRTFEPYFYALLKDDSAIEDVKKVTAKRHGTVVKVKRAEKVQKKFLGRPIEVWKLYFNHPQDVPAIRDRIRAHPAVVDIYEYDIPFAKRYLIDKGLIPMEGDEELKMLAFDIETLYHEGEEFAEGPILMISYADEEGARVITWKNVDLPYVDVVSTEREMIKRFLRVVKEKDPDVLITYNGDNFDFAYLKKRCEKLGINFALGRDGSEPKIQRMGDRFAVEVKGRIHFDLYPVIRRTINLPTYTLEAVYEAVFGQPKEKVYAEEITTAWETGENLERVARYSMEDAKVTYELGKEFLPMEAQLSRLVGQSLWDVSRSSTGNLVEWFLLRKAYKRNELAPNKPDEKELARRRQSYEGGYVKEPERGLWENIVYLDFRSIAPSIIITHNVSPDTLNREGCKEYDVAPQVGHRFCKDFPGFIPSLLGHLLEERQKIKTKMKETQDPIEKILLDYRQKAIKLLANSFYGYYGYARARWYCKECAESVTAWGREYITMTIKEIEEKYGFKVIYSDTDGFFATIPGADAETVKKKAMEFLKYINAKLPGALELEYEGFYKRGFFVTKKKYAVIDEEGKITTRGLEIVRRDWSEIAKETQARVLEAILKHGDVEEAVRIVKEVTEKLSKYEVPPEKLVIHEQITRDLRDYKATGPHVAVAKRLAARGVKIRPGTVISYIVLKGSGRIGDRAIPADEFDPTKHRYDAEYYIENQVLPAVERILKAFGYRKEDLRYQKTKQVGLGAWLKVKGKK

SEQ ID NO: 2 - protein, 778 aa, Artificial
  2
MASAILDTDYITENGKPVIRVFKKENGEFKIEYDRTFEPYFYALLKDDSAIEDVKKVTAKRHGTVVKVKRAEKVQKKFLGRPIEVWKLYFNHPQDVPAIRDRIRAHPAVVDIYEYDIPFAKRYLIDKGLIPMEGDEELKMLAFDIETLYHEGEEFAEGPILIISYADEEGARVITWKNVDLPYVDVVSTEREMIKRFLRVVKEKDPDVLITYNGDNFDFAYLKKRCEKLGINFALGRDGSEPKIQRMGDRFAVEVKGRIHFDLYPVIRRTINLPTYTLEAVYEAVFGQPKEKVYAEEITTAWETGENLERVARYSMEDAKVTYELGKEFLPMEAQLSRLVGQSLWDVSRSSTGNLVEWFLLRKAYKRNELAPNKPDEKELARRRQSYEGGYVKEPERGLWENIVYLDFRSIAPSIIITHNVSPDTLNREGCKEYDVAPQVGHRFCKDFPGFIPSLLGHLLEERQKIKTKMKETQDPIEKILLDYRQKAIKLLANSFYGYYGYARARWYCKECAESVTAWGREYITMTIKEIEEKYGFKVVYSDTDGFFATIPGADAETVKKKAMEFLKYINAKLPGALELEYEGFYKRGFFVTKKKYTVIDEEGKITTRGLEIVRRDWSEIAKETQARVLEAILKHGDVEEAVRIVKEVTEKLSKYEVPPEKLVIHEQITRDLRDYKATGPHVAVAKRLAARGVKIRPGTVISYIVLKGSGRIGDRAIPADEFDPTKQRYDAEYYIENQVLPAVERILKAFGYRKEDLRYQKTKQVGLGAWLKVKGKK

SEQ ID NO: 3 - protein, 778 aa, Artificial
  3
MASAILDTDYITENGKPVIRVFKKENGEFKIEYDRTYEPYFYALLKDVSAIEDVKKVTAKRHGTVVKVKRAEKVQKKFLGRPIEVWKLYFNHPQDVPAIHDRIRAHPAVVDIYEYDIPFAKRYLIDKGLIPMEGDEELKMLAFDIETLYHEGEAFAEGPILMISYADEEGARVITWKNVDLPYVDVVSTEREMIKRFLRVVKEKDPDVLITYNGDNFDFANLKKRCEKLGINFALGRDGSEPNILRMGDRFAVEVKGRIHFDLYPVIRRTTNLPTYTLEAVYEAVFGQPKEKVYAVEITTAWETGESLERVARYSMEDAKVTYELGKEFLPMEAQLSRLVGQSLWDVSRSSTGNLVEWFLLRKAYKRNELAPNKPDEKELARRRQSYEGGYVKEPERGLWENIVYLDFRSIAPSIIITHNVSPDTLNREGCKEYDVAPQVGHRFCKDFPGFIPSLLGHLLEERQKIKTKMKETQDPIEKILLDYRQKAIKLLANSFYGYYGYARARWYCKECAESVTAWGREYITMTIKEIEEKYGFKVIYSDTDGFFATIPGADAETVKKKAMEFLKYINAKLPGALELEYEGFYKRGFFVTKKKYAVIDEEGKITTRGLEIVRRDWSEIAKETQARVLEAILKHGDVEEAVRIVKEVTEKLSKYEVPPEKLVIHEQITRDLRDYKATGPHVAVAKRLAARGVKIRPGTVISYIVLKGSGRIGDRAIPADEFDPTKHRYDAEYYIENQVLPAVERILKAYGYRKEDQRYQKTKQIGLGAWLKVKGKK

SEQ ID NO: 4 - protein, 778 aa, Artificial
  4
MASAILDTDYITENGKPVIRVFKKENGEFKIEYDRTYEPYFYAQLKDVSAIEDVKKVTAKRHGTVVKVKRAEKVQKKFLGRPIEVWKLYFNHPQDVPAIHDRIRAHPAVVDIYEYDIPFAKRYLIDKGLIPMEGDEELKMLAFDIETLHHEGEAFAEGPILMISYADEEGARVITWKNVDLPYVDVVSTEREMIKRFLRVVKEKDPDVLITYNGDNFDFAYLKKRCEKLGINFALGRDGSEPNILRMGDRFAVEVKGRIHFDLYPVIRRTTNLPTYTLEAVYEAVFGQPKEKVYAVEITTAWETGESLERVARYSMEDAKVTYELGKEFLPMEAQLSRLVGQSLWDVSRSSTGNLVEWFLLRKAYKRNELAPNKPDEKELARRRQSYEGGYVKEPERGLWENIVYLDFRSIAPSIIITHNVSPDTLNREGCKEYDVAPQVGHRFCKDFPGFIPSLLGHLLEERQKIKTKMKETQDPIEKILLDYRQKAIKLLANSFYGYYGYARARWYCKECAESVTAWGREYITMTIKEIEEKYGFKVIYSDTDGFFATIPGADAETVKKKAMEFLKYINAKLPGALELEYEGFYKRGFFVTKKKYAVIDEEGKITTRGLEIVRRDWSEIAKETQARVLEAILKHGDVEEAVRIVKEVTEKLSKYEVPPEKLVIHEQITRDLRDYKATGPHVAVAKRLAARGVKIRPGTVISYIVLKGSGRIGDRAIPADEFDPTKHRYDAEYYIENQVLPAVERILKAYGYRKEDQRYQKTKQIGLGAWLKVKGKK

SEQ ID NO: 5 - protein, 778 aa, Artificial
  5
MASAILDTDYITENGKPVIRVFKKENGEFKIEYDRTYEPYFYALLKDVSAIEDVKKVTAKRHGTVVKVKRAEKVQKKFLGRPIEVWKLYFNHPQDVPAIHDRIRAHPAVVDIYEYDIPFAKRYLIDKGLIPMEGDEELKMLAFDIETLYHEGEAFAEGPILMISYADEEGARVITWKNVDLPYVDVVSTEREMIKCFLRVVKEKDPDVLITYNGDNHDFANLKKRCEKLGINFALGRDGSEPNILRMGDRFAVEVKGRIHFDLYPVIRRTTNLPTYTLEAVYEAVFGQPKEKVYAVEITTAWETGESLERVARYSMEDAKVTYELGKEFLPMEAQLSRLVGQSLWHVSRSSTGNLVEWFLLRKAYKRNELAPNKPDEKELARRRQSYEGGYVKEPERGLWENIVYLDFRSIAPSIIITHNVSPDTLNREGCKEYDVAPQVGHRFCKDFPGFIPSLLGHLLEERQKIKTKMKETQDPIEKILLDYRQKAIKLLANSFYGYYGYARARWYCKECAESVTAWGREYITMTIKEIEEKYGFKVIYSDTDGFFATIPGADAETVKKKAMEFLKYINAKLPGALELEYEGFYKRGFFVTKKKYAVIDEEGKITTRGLEIVRRDWSEIAKETQARVLEAILKHGDVEEAVRIVKEVTEKLSKYEVPPEKLVIHEQITRDLRDYKATGPHVAVAKRLAARGVKIRPGTVISYIVLKGSGRIGDRAIPADEFDPTKHRYDAEYYIENQVLPAVERILKAYGYRKEDQRYQKTKQIGLGAWLKVKGKK

SEQ ID NO: 6 - protein, 778 aa, Artificial
  6
MASAILDTDYITENGKPVIRVFKKENGEFKIEYDRTYEPYFYALLKDVSAIEDVKKVTAKRHGTVVKVKRAEKVQKKFLGRPIEVWKLYFNHPLDVPAIHDRIRAHPAVVDIYEYDIPFAKRYLIDKGLIPMEGDEELKMLAFDIETLYHEGEAFAEGPILMISYADEEGARVITWKNVDLPYVDVVSTEREMIKRFLRVVKEKDPDVLITYNGDNFDFANLKKRCEKLGINFALGRDGSEPNILRMGDRFAVEVKGRIHFDLYPVIRRTTNLPTYTLEAVYEAVFGQPKEKVYAVEITTAWETGESLERVARYSMEDAKVTYELGKEFLPMEAQLSRLVGQSLWDVSRSSTGNLVEWFLLRKAYKRNELAPNKPDEKELARRRQSYEGGYVKEPERGLWENIVYLDFRSIAPSIIITHNVSPDTLNREGCKEYDVAPQVGHRFCKDFPGFIPSLLGHLLEERQKIKTKMKETQDPIEKILLDYRQKAIKLLANSFYGYYGYARARWYCKECAESVTAWGREYITMTIKEIEEKYGFKVIYSDTDGFFATIPGADAETVKKKAMEFLKYINAKLPGALELEYEGFYKRGFFVTKKKYAVIDEEGKITTRGLEIVRRDWSEIAKETQARVLEAILKHGDVEEAVRIVKEVTEKLSKYEVPPEKLVIHEQITRDLRDYKATGPHVAVAKRLAARGVKIRPGTVISYIVLKGSGRIGDRAIPADEFDPTKHRYDAEYYIENQVLPAVERILKAYGYRKEDQRYQKTKQIGLGAWLKVKGKK

SEQ ID NO: 7 - protein, 778 aa, Artificial
  7
MASAILDTDYITENGKPVIRVFKKENGEFKIEYDRTFEPYFYALLKDDSAIEDVKKVTAKRHGTVVKVKRAEKVQKKFLGRPIEVWKLYFNHPQDVPAIRDRIRAHPAVVDIYEYDIPFAKRYLIDKGLIPMEGDEELKMLAFDIETLYHEGEAFAEGPILMISYADEEGARVITWKNVDLPYVDVVSTEREMIKRFLRVVKEKDPDVLITYNGDNFDFAYLKKRCEKLGINFALGRDGSEPKIQRMGDRFAVEVKGRIHFDLYPVIRRTINLPTYTLEAVYEAVFGQPKEKVYAVEITTAWETGESLERVARYSMEDAKVTYELGKEFLPMEAQLSRLVGQSLWDVSRSSTGNLVEWFLLRKAYKRNELAPNKPDEKELARRRQSYEGGYVKEPERGLWENIVYLDFRSIAPSIIITHNVSPDTLNREGCKEYDVAPQVGHRFCKDFPGFIPSLLGHLLEERQKIKTKMKETQDPIEKILLDYRQKAIKLLANSFYGYYGYARARWYCKECAESVTAWGREYITMTIKEIEEKYGFKVIYSDTDGFFATIPGADAETVKKKAMEFLKYINAKLPGALELEYEGFYKRGFFVTKKKYAVIDEEGKITTRGLEIVRRDWSEIAKETQARVLEAILKHGDVEEAVRIVKEVTEKLSKYEVPPEKLVIHEQITRDLRDYKATGPHVAVAKRLAARGVKIRPGTVISYIVLKGSGRIGDRAIPADEFDPTKHRYDAEYYIENQVLPAVERILKAYGYRKEDQRYQKTKQVGLGAWLKVKGKK

SEQ ID NO: 8 - protein, 778 aa, Artificial
  8
MASAILDTDYITENGKPVIRVFKKENGEFKIEYDRTYEPYFYALLKDVSAIEDVKKVTAKRHGTVVKVKRAEKVQKKFLGRPIEVWKLYFNHPHDVPAIHDRIRAHPAVVDIYEYDIPFAKRYLIDKGLIPMEGDEELKMLAFDIETLYHEGEAFAEGPILMISYADEEGARVITWKNVDLPYVDVVSTEREMIKRFLRVVKEKDPDVLITYNGDNFDFANLKKRCEKLGINFALGRDGSEPNILRMGDRFAVEVKGRIHFDLYPVIRRTTNLPTYTLEAVYEAVFGQPKEKVYAVEITTAWETGESLERVARYSMEDAKVTYELGKEFLPMEAQLSRLVGQSLWDVSRSSTGNLVEWFLLRKAYKRNELAPNKPDEKELARRRQSYEGGYVKEPERGLWENIVYLDFRSIAPSIIITHNVSPDTLNREGCKEYDVAPQVGHRFCKDFPGFIPSLLGHLLEERQKIKTKMKETQDPIEKILLDYRQKAIKLLANSFYGYYGYARARWYCKECAESVTAWGREYITMTIKEIEEKYGFKVIYSDTDGFFATIPGADAETVKKKAMEFLKYINAKLPGALELEYEGFYKRGFFVTKKKYAVIDEEGKITTRGLEIVRRDWSEIAKETQARVLEAILKHGDVEEAVRIVKEVTEKLSKYEVPPEKLVIHEQITRDLRDYKATGPHVAVAKRLAARGVKIRPGTVISYIVLKGSGRIGERAIPADEFDPTKQRYDAEYYIENQVLPAVERILKAYGYRKEDQRYQKTKQIGLGAWLKVKGKK

SEQ ID NO: 9 - protein, 778 aa, Artificial
  9
MASAILDTDYITENGKPVIRVFKKENGEFKIEYDRTYEPYFYALLKDVSAIEDVKKVTAKRHGTVVKVKRAEKVQKKFLGRPIEVWKLYFNHPLDVPAIHDRIRAHPAVVDIYEYDIPFAKRYLIDKGLIPMEGDEELKMLAFDIETLYHEGEAAAEGPILMISYADEEGARVITWKNVDLPYVDVVSTEREMIKRFLRVVKEKDPDVLITYNGDNFDFANLKKRCEKLGINFALGRDGSEPNILRMGDRFAVEVKGRIHFDLYPVIRRTTNLPTYTLEAVYEAVFGQPKEKVYAVEITTAWETGESLERVARYSMEDAKVTYELGKEFLPMEAQLSRLVGQSLWDVSRSSTGNLVEWFLLRKAYKRNELAPNKPDEKELARRRQSYEGGYVKEPERGLWENIVYLDFRSIAPSIIITHNVSPDTLNREGCKEYDVAPQVGHRFCKDFPGFIPSLLGHLLEERQKIKTKMKETQDPIEKILLDYRQKAIKLLANSFYGYYGYARARWYCKECAESVTAWGREYITMTIKEIEEKYGFKVIYSDTDGFFATIPGADAETVKKKAMEFLKYINAKLPGALELEYEGFYKRGFFVTKKKYAVIDEEGKITTRGLEIVRRDWSEIAKETQARVLEAILKHGDVEEAVRIVKEVTEKLSKYEVPPEKLVIHEQITRDLRDYKATGPHVAVAKRLAARGVKIRPGTVISYIVLKGSGRIGDRAIPADEFDPTKHRYDAEYYIENQVLPAVERILKAYGYRKEDQRYQKTKQIGLGAWLKVKGKK

SEQ ID NO: 10 - DNA, 2337 bp, Artificial
  10
atggcgagcgcgattctggacactgattacattaccgaaaacggtaaaccggttatccgcgtgttcaagaaagagaatggtgagttcaaaatcgagtacgatcgcacgtttgaaccgtacttctatgctctgctgaaagacgattctgcgattgaagatgtgaaaaaagtgacggcgaaacgtcacggcaccgtggttaaggtgaaacgtgcggagaaagtgcaaaagaaattcctgggccgtccgatcgaagtttggaagctgtactttaaccacccacaagacgtcccggcgattcgtgaccgcatccgtgcgcacccggctgtggttgacatctatgagtacgatattccgttcgctaagagatacttgattgacaagggtctgatccctatggaaggtgacgaagaactgaagatgctggcgttcgacatcgaaactctgtaccacgagggtgaagagtttgccgagggtccgatcttgatgatttcctacgcggacgaagagggcgcacgtgttatcacgtggaaaaatgttgatctgccgtatgttgacgtcgtaagcaccgagcgtgagatgatcaaacgttttctgcgcgttgttaaagaaaaagatcctgacgtgctgatcacctacaacggtgacaatttcgatttcgcgtacctgaagaaacgttgcgaaaaactgggtattaacttcgcgctgggtcgcgatggctctgaaccgaagatccagcgcatgggtgatcgttttgcggtcgaggtgaagggtcgcattcatttcgacctgtacccggtgattcgtcgtaccatcaacttgccgacttacaccctggaagccgtctatgaagctgtatttggtcaaccgaaagaaaaagtgtacgctgaggaaattacgacggcgtgggaaaccggtgagaacctggagcgcgttgcacgttattctatggaggacgcgaaagttacctacgaactgggtaaagagttcctgccgatggaggcccaactgtcccgtctggtgggccaaagcctgtgggacgtcagccgttcgtccaccggcaacttggttgaatggttcctgctgcgtaaggcatacaagcgtaacgaactggcgccgaataagccggacgagaaagaattggcgcgtcgccgccagagctatgagggtggttatgtcaaagaaccggagcgcggcttgtgggagaacatcgtctatttggattttcgtagcattgcaccgagcatcattatcacgcataatgtgagcccggatacgttgaatcgtgagggctgtaaggaatacgacgtggcgcctcaggttggccaccgtttctgcaaggactttccgggctttataccaagtctcttgggacatttgttagaggaaagacaaaagattaagacaaaaatgaaggaaactcaagatcctatagaaaaaatactccttgactatagacaaaaagcgataaaactcttagcaaattctttctacggatattatggctatgcgcgtgcgcgctggtattgcaaagagtgtgccgagagcgtgaccgcttggggtcgtgagtacattaccatgacgatcaaagagattgaagagaaatacggctttaaggttatctatagcgacaccgacggtttctttgcaactatccctggcgcagacgcagaaaccgttaagaaaaaggcaatggagtttctgaagtatatcaacgcgaagttgccaggcgccctggaactggagtacgagggcttctacaagcgtggctttttcgtgacgaagaagaagtacgcggtcattgacgaagagggcaagattacgacccgtggtctggaaattgttcgccgtgactggtccgagattgcgaaagaaacccaggcgagagtgctggaagcgattctgaagcatggtgatgtcgaggaagccgtgcgtatcgttaaagaagtgacggagaagttgagcaagtacgaagtcccaccggagaaactggtgattcatgagcagatcacgcgcgatttacgtgactataaagcaaccggtccgcatgttgccgtggcaaagcgtctggctgcgcgtggcgttaagatccgtccgggcacggttattagctacattgtgttgaaaggtagcggtcgtattggcgaccgcgccattccggccgacgagttcgatccgaccaagcaccgctacgatgcagagtattacatcgagaaccaagtgctgccggctgtagagcgtattctgaaggcattcggttatcgtaaagaagatctgcgctatcaaaagacgaaacaagttggcctgggtgcgtggctgaaggtcaagggcaagaaataa

SEQ ID NO: 11 - DNA, 2337 bp, Artificial
  11
atggcgagcgcgattctggacactgattacattaccgaaaacggtaaaccggttatccgcgtgttcaagaaagagaatggtgagttcaaaatcgagtacgatcgcacgtttgaaccgtacttctatgctctgctgaaagacgattctgcgattgaagatgtgaaaaaagtgacggcgaaacgtcacggcaccgtggttaaggtgaaacgtgcggagaaagtgcaaaagaaattcctgggccgtccgatcgaagtttggaagctgtactttaaccacccacaagacgtcccggcgattcgtgaccgcatccgtgcgcacccggctgtggttgacatctatgagtacgatattccgttcgctaagagatacttgattgacaagggtctgatccctatggaaggtgacgaagaactgaagatgctggcgttcgacatcgaaactctgtaccacgagggtgaagagtttgccgagggtccgatcttgatcatttcctacgcggacgaagagggcgcacgtgttatcacgtggaaaaatgttgatctgccgtatgttgacgtcgtaagcaccgagcgtgagatgatcaaacgttttctgcgcgttgttaaagaaaaagatcctgacgtgctgatcacctacaacggtgacaatttcgatttcgcgtacctgaagaaacgttgcgaaaaactgggtattaacttcgcgctgggtcgcgatggctctgaaccgaagatccagcgcatgggtgatcgttttgcggtcgaggtgaagggtcgcattcatttcgacctgtacccggtgattcgtcgtaccatcaacttgccgacttacaccctggaagccgtctatgaagctgtatttggtcaaccgaaagaaaaagtgtacgctgaggaaattacgacggcgtgggaaaccggtgagaacctggagcgcgttgcacgttattctatggaggacgcgaaagttacctacgaactgggtaaagagttcctgccgatggaggcccaactgtcccgtctggtgggccaaagcctgtgggacgtcagccgttcgtccaccggcaacttggttgaatggttcctgctgcgtaaggcatacaagcgtaacgaactggcgccgaataagccggacgagaaagaattggcgcgtcgccgccagagctatgagggtggttatgtcaaagaaccggagcgcggcttgtgggagaacatcgtctatttggattttcgtagcattgcaccgagcatcattatcacgcataatgtgagcccggatacgttgaatcgtgagggctgtaaggaatacgacgtggcgcctcaggttggccaccgtttctgcaaggactttccgggctttataccaagtctcttgggacatttgttagaggaaagacaaaagattaagacaaaaatgaaggaaactcaagatcctatagaaaaaatactccttgactatagacaaaaagcgataaaactcttagcaaattctttctacggatattatggctatgcgcgtgcgcgctggtattgcaaagagtgtgccgagagcgtgaccgcttggggtcgtgagtacattaccatgacgatcaaagagattgaagagaaatacggctttaaggttgtttatagcgacaccgacggtttctttgcaactatccctggcgcagacgcagaaaccgttaagaaaaaggcaatggagtttctgaagtatatcaacgcgaagttgccaggcgccctggaactggagtacgagggcttctacaagcgtggctttttcgtgacgaagaagaagtacacggtcattgacgaagagggcaagattacgacccgtggtctggaaattgttcgccgtgactggtccgagattgcgaaagaaacccaggcgagagtgctggaagcgattctgaagcatggtgatgtcgaggaagccgtgcgtatcgttaaagaagtgacggagaagttgagcaagtacgaagtcccaccggagaaactggtgattcatgagcagatcacgcgcgatttacgtgactataaagcaaccggtccgcatgttgccgtggcaaagcgtctggctgcgcgtggcgttaagatccgtccgggcacggttattagctacattgtgttgaaaggtagcggtcgtattggcgaccgcgccattccggccgacgagttcgatccgaccaagcaacgctacgatgcagagtattacatcgagaaccaagtgctgccggctgtagagcgtattctgaaggcattcggttatcgtaaagaagatctgcgctatcaaaagacgaaacaagttggcctgggtgcgtggctgaaggtcaagggcaagaaataa

SEQ ID NO: 12 - DNA, 2337 bp, Artificial
  12
atggcgagcgcgattctggacactgattacattaccgaaaacggtaaaccggttatccgcgtgttcaagaaagagaatggtgagttcaaaatcgagtacgatcgcacgtatgaaccgtacttctatgctctgctgaaagacgtttctgcgattgaagatgtgaaaaaagtgacggcgaaacgtcacggcaccgtggttaaggtgaaacgtgcggagaaagtgcaaaagaaattcctgggccgtccgatcgaagtttggaagctgtactttaaccacccacaagacgtcccggcgattcatgaccgcatccgtgcgcacccggctgtggttgacatctatgagtacgatattccgttcgctaagagatacttgattgacaagggtctgatccctatggaaggtgacgaagaactgaagatgctggcgttcgacatcgaaactctgtaccacgagggtgaagcgtttgccgagggtccgatcttgatgatttcctacgcggacgaagagggcgcacgtgttatcacgtggaaaaatgttgatctgccgtatgttgacgtcgtaagcaccgagcgtgagatgatcaaacgttttctgcgcgttgttaaagaaaaagatcctgacgtgctgatcacctacaacggtgacaatttcgatttcgcgaatctgaagaaacgttgcgaaaaactgggtattaacttcgcgctgggtcgcgatggctctgaaccgaatatcctgcgcatgggtgatcgttttgcggtcgaggtgaagggtcgcattcatttcgacctgtacccggtgattcgtcgtaccaccaacttgccgacttacaccctggaagccgtctatgaagctgtatttggtcaaccgaaagaaaaagtgtacgctgtggaaattacgacggcgtgggaaaccggtgagagcctggagcgcgttgcacgttattctatggaggacgcgaaagttacctacgaactgggtaaagagttcctgccgatggaggcccaactgtcccgtctggtgggccaaagcctgtgggacgtcagccgttcgtccaccggcaacttggttgaatggttcctgctgcgtaaggcatacaagcgtaacgaactggcgccgaataagccggacgagaaagaattggcgcgtcgccgccagagctatgagggtggttatgtcaaagaaccggagcgcggcttgtgggagaacatcgtctatttggattttcgtagcattgcaccgagcatcattatcacgcataatgtgagcccggatacgttgaatcgtgagggctgtaaggaatacgacgtggcgcctcaggttggccaccgtttctgcaaggactttccgggctttataccaagtctcttgggacatttgttagaggaaagacaaaagattaagacaaaaatgaaggaaactcaagatcctatagaaaaaatactccttgactatagacaaaaagcgataaaactcttagcaaattctttctacggatattatggctatgcgcgtgcgcgctggtattgcaaagagtgtgccgagagcgtgaccgcttggggtcgtgagtacattaccatgacgatcaaagagattgaagagaaatacggctttaaggttatctatagcgacaccgacggtttctttgcaactatccctggcgcagacgcagaaaccgttaagaaaaaggcaatggagtttctgaagtatatcaacgcgaagttgccaggcgccctggaactggagtacgagggcttctacaagcgtggctttttcgtgacgaagaagaagtacgcggtcattgacgaagagggcaagattacgacccgtggtctggaaattgttcgccgtgactggtccgagattgcgaaagaaacccaggcgagagtgctggaagcgattctgaagcatggtgatgtcgaggaagccgtgcgtatcgttaaagaagtgacggagaagttgagcaagtacgaagtcccaccggagaaactggtgattcatgagcagatcacgcgcgatttacgtgactataaagcaaccggtccgcatgttgccgtggcaaagcgtctggctgcgcgtggcgttaagatccgtccgggcacggttattagctacattgtgttgaaaggtagcggtcgtattggcgaccgcgccattccggccgacgagttcgatccgaccaagcaccgctacgatgcagagtattacatcgagaaccaagtgctgccggctgtagagcgtattctgaaggcatacggttatcgtaaagaagatcagcgctatcaaaagacgaaacaaattggcctgggtgcgtggctgaaggtcaagggcaagaaataa

SEQ ID NO: 13 - DNA, 2337 bp, Artificial
  13
atggcgagcgcgattctggacactgattacattaccgaaaacggtaaaccggttatccgcgtgttcaagaaagagaatggtgagttcaaaatcgagtacgatcgcacgtatgaaccgtacttctatgctcagctgaaagacgtttctgcgattgaagatgtgaaaaaagtgacggcgaaacgtcacggcaccgtggttaaggtgaaacgtgcggagaaagtgcaaaagaaattcctgggccgtccgatcgaagtttggaagctgtactttaaccacccacaagacgtcccggcgattcatgaccgcatccgtgcgcacccggctgtggttgacatctatgagtacgatattccgttcgctaagagatacttgattgacaagggtctgatccctatggaaggtgacgaagaactgaagatgctggcgttcgacatcgaaactctgcaccacgagggtgaagcgtttgccgagggtccgatcttgatgatttcctacgcggacgaagagggcgcacgtgttatcacgtggaaaaatgttgatctgccgtatgttgacgtcgtaagcaccgagcgtgagatgatcaaacgttttctgcgcgttgttaaagaaaaagatcctgacgtgctgatcacctacaacggtgacaatttcgatttcgcgtatctgaagaaacgttgcgaaaaactgggtattaacttcgcgctgggtcgcgatggctctgaaccgaatatcctgcgcatgggtgatcgttttgcggtcgaggtgaagggtcgcattcatttcgacctgtacccggtgattcgtcgtaccaccaacttgccgacttacaccctggaagccgtctatgaagctgtatttggtcaaccgaaagaaaaagtgtacgctgtggaaattacgacggcgtgggaaaccggtgagagcctggagcgcgttgcacgttattctatggaggacgcgaaagttacctacgaactgggtaaagagttcctgccgatggaggcccaactgtcccgtctggtgggccaaagcctgtgggacgtcagccgttcgtccaccggcaacttggttgaatggttcctgctgcgtaaggcatacaagcgtaacgaactggcgccgaataagccggacgagaaagaattggcgcgtcgccgccagagctatgagggtggttatgtcaaagaaccggagcgcggcttgtgggagaacatcgtctatttggattttcgtagcattgcaccgagcatcattatcacgcataatgtgagcccggatacgttgaatcgtgagggctgtaaggaatacgacgtggcgcctcaggttggccaccgtttctgcaaggactttccgggctttataccaagtctcttgggacatttgttagaggaaagacaaaagattaagacaaaaatgaaggaaactcaagatcctatagaaaaaatactccttgactatagacaaaaagcgataaaactcttagcaaattctttctacggatattatggctatgcgcgtgcgcgctggtattgcaaagagtgtgccgagagcgtgaccgcttggggtcgtgagtacattaccatgacgatcaaagagattgaagagaaatacggctttaaggttatctatagcgacaccgacggtttctttgcaactatccctggcgcagacgcagaaaccgttaagaaaaaggcaatggagtttctgaagtatatcaacgcgaagttgccaggcgccctggaactggagtacgagggcttctacaagcgtggctttttcgtgacgaagaagaagtacgcggtcattgacgaagagggcaagattacgacccgtggtctggaaattgttcgccgtgactggtccgagattgcgaaagaaacccaggcgagagtgctggaagcgattctgaagcatggtgatgtcgaggaagccgtgcgtatcgttaaagaagtgacggagaagttgagcaagtacgaagtcccaccggagaaactggtgattcatgagcagatcacgcgcgatttacgtgactataaagcaaccggtccgcatgttgccgtggcaaagcgtctggctgcgcgtggcgttaagatccgtccgggcacggttattagctacattgtgttgaaaggtagcggtcgtattggcgaccgcgccattccggccgacgagttcgatccgaccaagcaccgctacgatgcagagtattacatcgagaaccaagtgctgccggctgtagagcgtattctgaaggcatacggttatcgtaaagaagatcagcgctatcaaaagacgaaacaaattggcctgggtgcgtggctgaaggtcaagggcaagaaataa

SEQ ID NO: 14 - DNA, 2337 bp, Artificial
  14
atggcgagcgcgattctggacactgattacattaccgaaaacggtaaaccggttatccgcgtgttcaagaaagagaatggtgagttcaaaatcgagtacgatcgcacgtatgaaccgtacttctatgctctgctgaaagacgtttctgcgattgaagatgtgaaaaaagtgacggcgaaacgtcacggcaccgtggttaaggtgaaacgtgcggagaaagtgcaaaagaaattcctgggccgtccgatcgaagtttggaagctgtactttaaccacccacaagacgtcccggcgattcatgaccgcatccgtgcgcacccggctgtggttgacatctatgagtacgatattccgttcgctaagagatacttgattgacaagggtctgatccctatggaaggtgacgaagaactgaagatgctggcgttcgacatcgaaactctgtaccacgagggtgaagcgtttgccgagggtccgatcttgatgatttcctacgcggacgaagagggcgcacgtgttatcacgtggaaaaatgttgatctgccgtatgttgacgtcgtaagcaccgagcgtgagatgatcaaatgttttctgcgcgttgttaaagaaaaagatcctgacgtgctgatcacctacaacggtgacaatcacgatttcgcgaatctgaagaaacgttgcgaaaaactgggtattaacttcgcgctgggtcgcgatggctctgaaccgaatatcctgcgcatgggtgatcgttttgcggtcgaggtgaagggtcgcattcatttcgacctgtacccggtgattcgtcgtaccaccaacttgccgacttacaccctggaagccgtctatgaagctgtatttggtcaaccgaaagaaaaagtgtacgctgtggaaattacgacggcgtgggaaaccggtgagagcctggagcgcgttgcacgttattctatggaggacgcgaaagttacctacgaactgggtaaagagttcctgccgatggaggcccaactgtcccgtctggtgggccaaagcctgtggcacgtcagccgttcgtccaccggcaacttggttgaatggttcctgctgcgtaaggcatacaagcgtaacgaactggcgccgaataagccggacgagaaagaattggcgcgtcgccgccagagctatgagggtggttatgtcaaagaaccggagcgcggcttgtgggagaacatcgtctatttggattttcgtagcattgcaccgagcatcattatcacgcataatgtgagcccggatacgttgaatcgtgagggctgtaaggaatacgacgtggcgcctcaggttggccaccgtttctgcaaggactttccgggctttataccaagtctcttgggacatttgttagaggaaagacaaaagattaagacaaaaatgaaggaaactcaagatcctatagaaaaaatactccttgactatagacaaaaagcgataaaactcttagcaaattctttctacggatattatggctatgcgcgtgcgcgctggtattgcaaagagtgtgccgagagcgtgaccgcttggggtcgtgagtacattaccatgacgatcaaagagattgaagagaaatacggctttaaggttatctatagcgacaccgacggtttctttgcaactatccctggcgcagacgcagaaaccgttaagaaaaaggcaatggagtttctgaagtatatcaacgcgaagttgccaggcgccctggaactggagtacgagggcttctacaagcgtggctttttcgtgacgaagaagaagtacgcggtcattgacgaagagggcaagattacgacccgtggtctggaaattgttcgccgtgactggtccgagattgcgaaagaaacccaggcgagagtgctggaagcgattctgaagcatggtgatgtcgaggaagccgtgcgtatcgttaaagaagtgacggagaagttgagcaagtacgaagtcccaccggagaaactggtgattcatgagcagatcacgcgcgatttacgtgactataaagcaaccggtccgcatgttgccgtggcaaagcgtctggctgcgcgtggcgttaagatccgtccgggcacggttattagctacattgtgttgaaaggtagcggtcgtattggcgaccgcgccattccggccgacgagttcgatccgaccaagcaccgctacgatgcagagtattacatcgagaaccaagtgctgccggctgtagagcgtattctgaaggcatacggttatcgtaaagaagatcagcgctatcaaaagacgaaacaaattggcctgggtgcgtggctgaaggtcaagggcaagaaataa

SEQ ID NO: 15 - DNA, 2337 bp, Artificial
  15
atggcgagcgcgattctggacactgattacattaccgaaaacggtaaaccggttatccgcgtgttcaagaaagagaatggtgagttcaaaatcgagtacgatcgcacgtatgaaccgtacttctatgctctgctgaaagacgtttctgcgattgaagatgtgaaaaaagtgacggcgaaacgtcacggcaccgtggttaaggtgaaacgtgcggagaaagtgcaaaagaaattcctgggccgtccgatcgaagtttggaagctgtactttaaccacccactggacgtcccggcgattcatgaccgcatccgtgcgcacccggctgtggttgacatctatgagtacgatattccgttcgctaagagatacttgattgacaagggtctgatccctatggaaggtgacgaagaactgaagatgctggcgttcgacatcgaaactctgtaccacgagggtgaagcgtttgccgagggtccgatcttgatgatttcctacgcggacgaagagggcgcacgtgttatcacgtggaaaaatgttgatctgccgtatgttgacgtcgtaagcaccgagcgtgagatgatcaaacgttttctgcgcgttgttaaagaaaaagatcctgacgtgctgatcacctacaacggtgacaatttcgatttcgcgaatctgaagaaacgttgcgaaaaactgggtattaacttcgcgctgggtcgcgatggctctgaaccgaatatcctgcgcatgggtgatcgttttgcggtcgaggtgaagggtcgcattcatttcgacctgtacccggtgattcgtcgtaccaccaacttgccgacttacaccctggaagccgtctatgaagctgtatttggtcaaccgaaagaaaaagtgtacgctgtggaaattacgacggcgtgggaaaccggtgagagcctggagcgcgttgcacgttattctatggaggacgcgaaagttacctacgaactgggtaaagagttcctgccgatggaggcccaactgtcccgtctggtgggccaaagcctgtgggacgtcagccgttcgtccaccggcaacttggttgaatggttcctgctgcgtaaggcatacaagcgtaacgaactggcgccgaataagccggacgagaaagaattggcgcgtcgccgccagagctatgagggtggttatgtcaaagaaccggagcgcggcttgtgggagaacatcgtctatttggattttcgtagcattgcaccgagcatcattatcacgcataatgtgagcccggatacgttgaatcgtgagggctgtaaggaatacgacgtggcgcctcaggttggccaccgtttctgcaaggactttccgggctttataccaagtctcttgggacatttgttagaggaaagacaaaagattaagacaaaaatgaaggaaactcaagatcctatagaaaaaatactccttgactatagacaaaaagcgataaaactcttagcaaattctttctacggatattatggctatgcgcgtgcgcgctggtattgcaaagagtgtgccgagagcgtgaccgcttggggtcgtgagtacattaccatgacgatcaaagagattgaagagaaatacggctttaaggttatctatagcgacaccgacggtttctttgcaactatccctggcgcagacgcagaaaccgttaagaaaaaggcaatggagtttctgaagtatatcaacgcgaagttgccaggcgccctggaactggagtacgagggcttctacaagcgtggctttttcgtgacgaagaagaagtacgcggtcattgacgaagagggcaagattacgacccgtggtctggaaattgttcgccgtgactggtccgagattgcgaaagaaacccaggcgagagtgctggaagcgattctgaagcatggtgatgtcgaggaagccgtgcgtatcgttaaagaagtgacggagaagttgagcaagtacgaagtcccaccggagaaactggtgattcatgagcagatcacgcgcgatttacgtgactataaagcaaccggtccgcatgttgccgtggcaaagcgtctggctgcgcgtggcgttaagatccgtccgggcacggttattagctacattgtgttgaaaggtagcggtcgtattggcgaccgcgccattccggccgacgagttcgatccgaccaagcaccgctacgatgcagagtattacatcgagaaccaagtgctgccggctgtagagcgtattctgaaggcatacggttatcgtaaagaagatcagcgctatcaaaagacgaaacaaattggcctgggtgcgtggctgaaggtcaagggcaagaaataa

SEQ ID NO: 16 - DNA, 2337 bp, Artificial
  16
atggcgagcgcgattctggacactgattacattaccgaaaacggtaaaccggttatccgcgtgttcaagaaagagaatggtgagttcaaaatcgagtacgatcgcacgtttgaaccgtacttctatgctctgctgaaagacgattctgcgattgaagatgtgaaaaaagtgacggcgaaacgtcacggcaccgtggttaaggtgaaacgtgcggagaaagtgcaaaagaaattcctgggccgtccgatcgaagtttggaagctgtactttaaccacccacaagacgtcccggcgattcgtgaccgcatccgtgcgcacccggctgtggttgacatctatgagtacgatattccgttcgctaagagatacttgattgacaagggtctgatccctatggaaggtgacgaagaactgaagatgctggcgttcgacatcgaaactctgtaccacgagggtgaagcgtttgccgagggtccgatcttgatgatttcctacgcggacgaagagggcgcacgtgttatcacgtggaaaaatgttgatctgccgtatgttgacgtcgtaagcaccgagcgtgagatgatcaaacgttttctgcgcgttgttaaagaaaaagatcctgacgtgctgatcacctacaacggtgacaatttcgatttcgcgtacctgaagaaacgttgcgaaaaactgggtattaacttcgcgctgggtcgcgatggctctgaaccgaagatccagcgcatgggtgatcgttttgcggtcgaggtgaagggtcgcattcatttcgacctgtacccggtgattcgtcgtaccatcaacttgccgacttacaccctggaagccgtctatgaagctgtatttggtcaaccgaaagaaaaagtgtacgctgtggaaattacgacggcgtgggaaaccggtgagagcctggagcgcgttgcacgttattctatggaggacgcgaaagttacctacgaactgggtaaagagttcctgccgatggaggcccaactgtcccgtctggtgggccaaagcctgtgggacgtcagccgttcgtccaccggcaacttggttgaatggttcctgctgcgtaaggcatacaagcgtaacgaactggcgccgaataagccggacgagaaagaattggcgcgtcgccgccagagctatgagggtggttatgtcaaagaaccggagcgcggcttgtgggagaacatcgtctatttggattttcgtagcattgcaccgagcatcattatcacgcataatgtgagcccggatacgttgaatcgtgagggctgtaaggaatacgacgtggcgcctcaggttggccaccgtttctgcaaggactttccgggctttataccaagtctcttgggacatttgttagaggaaagacaaaagattaagacaaaaatgaaggaaactcaagatcctatagaaaaaatactccttgactatagacaaaaagcgataaaactcttagcaaattctttctacggatattatggctatgcgcgtgcgcgctggtattgcaaagagtgtgccgagagcgtgaccgcttggggtcgtgagtacattaccatgacgatcaaagagattgaagagaaatacggctttaaggttatctatagcgacaccgacggtttctttgcaactatccctggcgcagacgcagaaaccgttaagaaaaaggcaatggagtttctgaagtatatcaacgcgaagttgccaggcgccctggaactggagtacgagggcttctacaagcgtggctttttcgtgacgaagaagaagtacgcggtcattgacgaagagggcaagattacgacccgtggtctggaaattgttcgccgtgactggtccgagattgcgaaagaaacccaggcgagagtgctggaagcgattctgaagcatggtgatgtcgaggaagccgtgcgtatcgttaaagaagtgacggagaagttgagcaagtacgaagtcccaccggagaaactggtgattcatgagcagatcacgcgcgatttacgtgactataaagcaaccggtccgcatgttgccgtggcaaagcgtctggctgcgcgtggcgttaagatccgtccgggcacggttattagctacattgtgttgaaaggtagcggtcgtattggcgaccgcgccattccggccgacgagttcgatccgaccaagcaccgctacgatgcagagtattacatcgagaaccaagtgctgccggctgtagagcgtattctgaaggcatacggttatcgtaaagaagatcagcgctatcaaaagacgaaacaagttggcctgggtgcgtggctgaaggtcaagggcaagaaataa

SEQ ID NO: 17 - DNA, 2337 bp, Artificial
  17
atggcgagcgcgattctggacactgattacattaccgaaaacggtaaaccggttatccgcgtgttcaagaaagagaatggtgagttcaaaatcgagtacgatcgcacgtatgaaccgtacttctatgctctgctgaaagacgtttctgcgattgaagatgtgaaaaaagtgacggcgaaacgtcacggcaccgtggttaaggtgaaacgtgcggagaaagtgcaaaagaaattcctgggccgtccgatcgaagtttggaagctgtactttaaccacccacacgacgtcccggcgattcatgaccgcatccgtgcgcacccggctgtggttgacatctatgagtacgatattccgttcgctaagagatacttgattgacaagggtctgatccctatggaaggtgacgaagaactgaagatgctggcgttcgacatcgaaactctgtaccacgagggtgaagcgtttgccgagggtccgatcttgatgatttcctacgcggacgaagagggcgcacgtgttatcacgtggaaaaatgttgatctgccgtatgttgacgtcgtaagcaccgagcgtgagatgatcaaacgttttctgcgcgttgttaaagaaaaagatcctgacgtgctgatcacctacaacggtgacaatttcgatttcgcgaatctgaagaaacgttgcgaaaaactgggtattaacttcgcgctgggtcgcgatggctctgaaccgaatatcctgcgcatgggtgatcgttttgcggtcgaggtgaagggtcgcattcatttcgacctgtacccggtgattcgtcgtaccaccaacttgccgacttacaccctggaagccgtctatgaagctgtatttggtcaaccgaaagaaaaagtgtacgctgtggaaattacgacggcgtgggaaaccggtgagagcctggagcgcgttgcacgttattctatggaggacgcgaaagttacctacgaactgggtaaagagttcctgccgatggaggcccaactgtcccgtctggtgggccaaagcctgtgggacgtcagccgttcgtccaccggcaacttggttgaatggttcctgctgcgtaaggcatacaagcgtaacgaactggcgccgaataagccggacgagaaagaattggcgcgtcgccgccagagctatgagggtggttatgtcaaagaaccggagcgcggcttgtgggagaacatcgtctatttggattttcgtagcattgcaccgagcatcattatcacgcataatgtgagcccggatacgttgaatcgtgagggctgtaaggaatacgacgtggcgcctcaggttggccaccgtttctgcaaggactttccgggctttataccaagtctcttgggacatttgttagaggaaagacaaaagattaagacaaaaatgaaggaaactcaagatcctatagaaaaaatactccttgactatagacaaaaagcgataaaactcttagcaaattctttctacggatattatggctatgcgcgtgcgcgctggtattgcaaagagtgtgccgagagcgtgaccgcttggggtcgtgagtacattaccatgacgatcaaagagattgaagagaaatacggctttaaggttatctatagcgacaccgacggtttctttgcaactatccctggcgcagacgcagaaaccgttaagaaaaaggcaatggagtttctgaagtatatcaacgcgaagttgccaggcgccctggaactggagtacgagggcttctacaagcgtggctttttcgtgacgaagaagaagtacgcggtcattgacgaagagggcaagattacgacccgtggtctggaaattgttcgccgtgactggtccgagattgcgaaagaaacccaggcgagagtgctggaagcgattctgaagcatggtgatgtcgaggaagccgtgcgtatcgttaaagaagtgacggagaagttgagcaagtacgaagtcccaccggagaaactggtgattcatgagcagatcacgcgcgatttacgtgactataaagcaaccggtccgcatgttgccgtggcaaagcgtctggctgcgcgtggcgttaagatccgtccgggcacggttattagctacattgtgttgaaaggtagcggtcgtattggcgagcgcgccattccggccgacgagttcgatccgaccaagcaacgctacgatgcagagtattacatcgagaaccaagtgctgccggctgtagagcgtattctgaaggcatacggttatcgtaaagaagatcagcgctatcaaaagacgaaacaaattggcctgggtgcgtggctgaaggtcaagggcaagaaataa

SEQ ID NO: 18 - DNA, 2337 bp, Artificial
  18
atggcgagcgcgattctggacactgattacattaccgaaaacggtaaaccggttatccgcgtgttcaagaaagagaatggtgagttcaaaatcgagtacgatcgcacgtatgaaccgtacttctatgctctgctgaaagacgtttctgcgattgaagatgtgaaaaaagtgacggcgaaacgtcacggcaccgtggttaaggtgaaacgtgcggagaaagtgcaaaagaaattcctgggccgtccgatcgaagtttggaagctgtactttaaccacccactggacgtcccggcgattcatgaccgcatccgtgcgcacccggctgtggttgacatctatgagtacgatattccgttcgctaagagatacttgattgacaagggtctgatccctatggaaggtgacgaagaactgaagatgctggcgttcgacatcgaaactctgtaccacgagggtgaagcggctgccgagggtccgatcttgatgatttcctacgcggacgaagagggcgcacgtgttatcacgtggaaaaatgttgatctgccgtatgttgacgtcgtaagcaccgagcgtgagatgatcaaacgttttctgcgcgttgttaaagaaaaagatcctgacgtgctgatcacctacaacggtgacaatttcgatttcgcgaatctgaagaaacgttgcgaaaaactgggtattaacttcgcgctgggtcgcgatggctctgaaccgaatatcctgcgcatgggtgatcgttttgcggtcgaggtgaagggtcgcattcatttcgacctgtacccggtgattcgtcgtaccaccaacttgccgacttacaccctggaagccgtctatgaagctgtatttggtcaaccgaaagaaaaagtgtacgctgtggaaattacgacggcgtgggaaaccggtgagagcctggagcgcgttgcacgttattctatggaggacgcgaaagttacctacgaactgggtaaagagttcctgccgatggaggcccaactgtcccgtctggtgggccaaagcctgtgggacgtcagccgttcgtccaccggcaacttggttgaatggttcctgctgcgtaaggcatacaagcgtaacgaactggcgccgaataagccggacgagaaagaattggcgcgtcgccgccagagctatgagggtggttatgtcaaagaaccggagcgcggcttgtgggagaacatcgtctatttggattttcgtagcattgcaccgagcatcattatcacgcataatgtgagcccggatacgttgaatcgtgagggctgtaaggaatacgacgtggcgcctcaggttggccaccgtttctgcaaggactttccgggctttataccaagtctcttgggacatttgttagaggaaagacaaaagattaagacaaaaatgaaggaaactcaagatcctatagaaaaaatactccttgactatagacaaaaagcgataaaactcttagcaaattctttctacggatattatggctatgcgcgtgcgcgctggtattgcaaagagtgtgccgagagcgtgaccgcttggggtcgtgagtacattaccatgacgatcaaagagattgaagagaaatacggctttaaggttatctatagcgacaccgacggtttctttgcaactatccctggcgcagacgcagaaaccgttaagaaaaaggcaatggagtttctgaagtatatcaacgcgaagttgccaggcgccctggaactggagtacgagggcttctacaagcgtggctttttcgtgacgaagaagaagtacgcggtcattgacgaagagggcaagattacgacccgtggtctggaaattgttcgccgtgactggtccgagattgcgaaagaaacccaggcgagagtgctggaagcgattctgaagcatggtgatgtcgaggaagccgtgcgtatcgttaaagaagtgacggagaagttgagcaagtacgaagtcccaccggagaaactggtgattcatgagcagatcacgcgcgatttacgtgactataaagcaaccggtccgcatgttgccgtggcaaagcgtctggctgcgcgtggcgttaagatccgtccgggcacggttattagctacattgtgttgaaaggtagcggtcgtattggcgaccgcgccattccggccgacgagttcgatccgaccaagcaccgctacgatgcagagtattacatcgagaaccaagtgctgccggctgtagagcgtattctgaaggcatacggttatcgtaaagaagatcagcgctatcaaaagacgaaacaaattggcctgggtgcgtggctgaaggtcaagggcaagaaataa

SEQ ID NO: 19 - protein, 775 aa, Artificial
  19
MILDTDYITENGKPVIRVFKKENGEFKIEYDRTFEPYFYALLKDDSAIEDVKKVTAKRHGTVVKVKRAEKVQKKFLGRPIEVWKLYFNHPQDVPAIRDRIRAHPAVVDIYEYDIPFAKRYLIDKGLIPMEGDEELTMLAFDIETLYHEGEEFGTGPILMISYADGSEARVITWKKIDLPYVDVVSTEKEMIKRFLRVVREKDPDVLITYNGDNFDFAYLKKRCEELGIKFTLGRDGSEPKIQRMGDRFAVEVKGRIHFDLYPVIRRTINLPTYTLEAVYEAVFGKPKEKVYAEEIAQAWESGEGLERVARYSMEDAKVTYELGREFFPMEAQLSRLIGQSLWDVSRSSTGNLVEWFLLRKAYKRNELAPNKPDERELARRRGGYAGGYVKEPERGLWDNIVYLDFRSLYPSIIITHNVSPDTLNREGCKEYDVAPEVGHKFCKDFPGFIPSLLGDLLEERQKIKRKMKATVDPLEKKLLDYRQRAIKILANSFYGYYGYAKARWYCKECAESVTAWGREYIEMVIRELEEKFGFKVLYADTDGLHATIPGADAETVKKKAKEFLKYINPKLPGLLELEYEGFYVRGFFVTKKKYAVIDEEGKITTRGLEIVRRDWSEIAKETQARVLEAILKHGDVEEAVRIVKEVTEKLSKYEVPPEKLVIHEQITRDLRDYKATGPHVAVAKRLAARGVKIRPGTVISYIVLKGSGRIGDRAIPADEFDPTKHRYDAEYYIENQVLPAVERILKAFGYRKEDLRYQKTKQVGLGAWLKVKGKK

SEQ ID NO: 20 - protein, 774 aa, Artificial
  20
MILDTDYITEDGKPVIRIFKKENGEFKIEYDRTFEPYFYALLKDDSAIEEVKKITAERHGTVVTVKRVEKVQKKFLGRPVEVWKLYFTHPQDVPAIRDKIREHPAVIDIYEYDIPFAKRYLIDKGLVPMEGDEELKMLAFDIETLYHEGEEFAEGPILMISYADEEGARVITWKNVDLPYVDVVSTEREMIKRFLRVVKEKDPDVLITYNGDNFDFAYLKKRCEKLGINFALGRDGSEPKIQRMGDRFAVEVKGRIHFDLYPVIRRTINLPTYTLEAVYEAVFGQPKEKVYAEEITTAWETGENLERVARYSMEDAKVTYELGKEFLPMEAQLSRLVGQSLWDVSRSSTGNLVEWFLLRKAYERNELAPNKPDEKELARRRQSYEGGYVKEPERGLWENIVYLDFRSIAPSIIITHNVSPDTLNREGCKEYDVAPQVGHRFCKDFPGFIPSLLGDLLEERQKIKKKMKATIDPIERKLLDYRQRAIKILANSYYGYYGYARARWYCKECAESVTAWGREYITMTIKEIEEKYGFKVIYSDTDGFFATIPGADAETVKKKAMEFLKYINAKLPGALELEYEGFYKRGFFVTKKKYAVIDEEGKITTRGLEIVRRDWSEIAKETQARVLEALLKDGDVEKAVRIVKEVTEKLSKYEVPPEKLVIHEQITRDLKDYKATGPHVAVAKRLAARGVKIRPGTVISYIVLKGSGRIGDRAIPFDEFDPTKHKYDAEYYIENQVLPAVERILRAFGYRKEDLRYQKTRQVGLSAWLKPKGT

SEQ ID NO: 21 - protein, 775 aa, Artificial
  21
MILDVDYITEEGKPVIRLFKKENGKFKIEHDRTFRPYIYALLRDDSKIEEVKKITGERHGKIVRIVDVEKVEKKFLGKPITVWKLYLEHPQDVPTLREKVREHPAVVDIFEYDIPFAKRYLIDKGLIPMEGEEELKILAFDIETLYHEGEEFGKGPIIMISYADENEARVITWKNIDLPYVESVSTEKEMIKRFLRIIREKDPDIIVTYNGDSFDFPYLAKRAEKLGIKLTIGRDGSEPKMQRIGDMTAVEVKGRIHFDLYHVIRTTINLPTYTLEAVYEAIFGKPKEKVYADEIAKAWESGENLERVAKYSMEDAKATYELGKEFLPMEIQLSRLVGQPLWDVSRSSTGNLVEWFLLRKAYERNEVAPNKPSEEEYQRRLRESYTGGFVKEPEKGLWENIVYLDYKSLYPSIIITHNVSPDTLNLEGCKNYDIAPQVGHKFCKDIPGFIPSLLGHLLEERQKIKTKMKETQDPIEKILLDYRQKAIKLLANSFYGYYGYAKARWYCKECAESVTAWGRKYIELVWKELEEKFGFKVLYIDTDGLYATIPGGESEEIKKKALEFVKYINSKLPGLLELEYEGFYKRGFFVTKKRYAVIDEEGKVITRGLEIVRRDWSEIAKETQARVLETILKHGDVEEAVRIVKEVIQKLANYEIPPEKLAIYEQITRPLHEYKAIGPHVAVAKKLAAKGVKIKPGMVIGYIVLRGDGPISNRAILAEEYDPKKHKYDAEYYIENQVLPAVLRILEGFGYRKEDLRYQKTRQVGLTSWLNIKKS

SEQ ID NO: 22 - DNA, 2328 bp, Artificial
  22
atgattctggacactgattacattaccgaaaacggtaaaccggttatccgcgtgttcaagaaagagaatggtgagttcaaaatcgagtacgatcgcacgtttgaaccgtacttctatgctctgctgaaagacgattctgcgattgaagatgtgaaaaaagtgacggcgaaacgtcacggcaccgtggttaaggtgaaacgtgcggagaaagtgcaaaagaaattcctgggccgtccgatcgaagtttggaagctgtactttaaccacccacaagacgtcccggcgattcgtgaccgcatccgtgcgcacccggctgtggttgacatctatgagtacgatattccgttcgctaagagatacttgattgacaagggtctgatccctatggaaggcgacgaagaactgaccatgctggccttcgatatcgagacgttgtatcacgagggcgaagagtttggcaccggcccaatcctgatgattagctatgccgacggttccgaagcgcgtgtgatcacctggaagaaaattgatctgccgtacgtcgatgtggtgagcacggaaaaagaaatgatcaaacgttttctgcgtgtggtccgtgagaaagatccggatgtcctgattacgtataacggtgacaattttgattttgcgtacctgaaaaagcgctgcgaggaactgggtatcaagttcacgctgggtcgtgatggtagcgagccgaagattcagcgtatgggtgaccgttttgcagttgaggtgaagggtcgcattcacttcgacctgtacccggttattcgccgcaccatcaacttgcctacctacaccctggaagcggtctatgaagctgtctttggcaaaccgaaagagaaagtttacgcggaagagatcgcgcaggcgtgggagagcggtgagggtctggaacgtgttgcccgctacagcatggaagatgcgaaggtgacttatgagttgggtcgcgagtttttcccgatggaagcacagctgagccgtctgatcggccaaagcctgtgggacgtcagccgttcgtccaccggcaacttggttgaatggttcctgctgcgtaaggcatacaagcgtaacgaactggcgccgaataagccggacgagcgtgagctggcccgtcgccgtggtggttatgccggtggctatgttaaagagccggagcgcggtctgtgggacaatatcgtgtatctggacttccgctccctgtatccgagcatcattatcacccacaatgttagcccggatactttaaaccgcgagggttgtaaagagtacgacgtggcgcctgaggtcggccacaagttttgcaaagatttcccgggcttcatcccaagcctgctgggcgatctgctggaggaacgtcagaagatcaaacgcaaaatgaaagcaacggttgatccgctggagaaaaagctgctggattatcgtcagcgcgcaattaagatcctggcgaatagcttttatggttactacggttatgccaaagcgcgttggtactgtaaagaatgcgctgagtctgtcaccgcgtggggccgtgagtacatcgaaatggttatccgtgagctcgaagagaaattcggttttaaggttctgtatgccgacaccgacggtctgcacgcgaccatcccgggtgcagacgccgaaaccgtcaagaagaaagcaaaagaatttctgaaatacattaatccgaaattgccgggtctgttggagttggagtatgagggtttctacgttcgtggcttctttgttaccaagaagaagtacgcggtcattgacgaagagggcaagattacgacccgtggtctggaaattgttcgccgtgactggtccgagattgcgaaagaaacccaggcgagagtgctggaagcgattctgaagcatggtgatgtcgaggaagccgtgcgtatcgttaaagaagtgacggagaagttgagcaagtacgaagtcccaccggagaaactggtgattcatgagcagatcacgcgcgatttacgtgactataaagcaaccggtccgcatgttgccgtggcaaagcgtctggctgcgcgtggcgttaagatccgtccgggcacggttattagctacattgtgttgaaaggtagcggtcgtattggcgaccgcgccattccggccgacgagttcgatccgaccaagcaccgctacgatgcagagtattacatcgagaaccaagtgctgccggctgtagagcgtattctgaaggcattcggttatcgtaaagaagatctgcgctatcaaaagacgaaacaagttggcctgggtgcgtggctgaaggtcaagggcaagaaataa

SEQ ID NO: 23 - DNA, 2328 bp, Artificial
  23
atgattttagatgtggattacataactgaagaaggaaaacctgttattaggctattcaaaaaagagaacggaaaatttaagatagagcatgatagaacttttagaccatacatttacgctcttctcagggatgattcaaagattgaagaagttaagaaaataacgggggaaaggcatggaaagattgtgagaattgttgatgtagagaaggttgagaaaaagtttctcggcaagcctattaccgtgtggaaactttatttggaacatccccaagatgttcccactttaagagaaaaagttagagaacatccagcagttgtggacatcttcgaatacgatattccatttgcaaagagatacctcatcgacaaaggcctaataccaatggagggggaagaagagctaaagattcttgccttcgatatagaaaccctctatcacgaaggagaagagtttggaaaaggcccaattataatgattagttatgcagatgaaaatgaagcaagggtgattacttggaaaaacatagatcttccatacgttgagtcagtatcaaccgagaaagagatgataaagagatttctcaggattatcagggagaaggatcctgacattatagttacttataatggagactcattcgacttcccatatttagcgaaaagggcagaaaaacttgggattaaattaaccattggaagagatggaagcgagcccaagatgcagagaataggcgatatgacggctgtagaagtcaagggaagaatacatttcgacttgtatcatgtaataaggacaacaataaatctcccaacatacacactagaggctgtatatgaagcaatttttggaaagccaaaggagaaggtatacgccgacgagatagcaaaagcctgggaaagtggagagaaccttgagagagttgccaaatactcgatggaagatgcaaaggcaacttatgaactcgggaaagaattccttccaatggaaattcagctttcaagattagttggacaacctttatgggatgtttcaaggtcaagcacagggaaccttgtagagtggttcttacttaggaaagcctacgaaagaaacgaagtagctccaaacaagccaagtgaagaggagtatcaaagaaggctcagggagagctacacaggtggattcgttaaagagccagaaaaggggttgtgggaaaacatagtatacctagattacaaatcactatatccctcgattataattacccacaatgtttctcccgatactctaaatcttgagggatgcaagaactatgatatcgctcctcaagtaggccacaagttctgcaaggacatccctggttttataccaagtctcttgggacatttgttagaggaaagacaaaagattaagacaaaaatgaaggaaactcaagatcctatagaaaaaatactccttgactatagacaaaaagcgataaaactcttagcaaattctttctacggatattatggctatgcaaaagcaagatggtactgtaaggagtgtgctgagagcgttactgcctggggaagaaagtacatcgagttagtatggaaggagctcgaagaaaagtttggatttaaagtcctctacattgacactgatggtctctatgcaactatcccaggaggagaaagtgaggaaataaagaaaaaggctctagaatttgtaaaatacataaattcaaagctccctggactgctagagcttgaatatgaagggttttataagaggggattcttcgttacgaagaagaggtatgcagtaatagatgaagaaggaaaagtcattactcgtggtttagagatagttaggagagattggagtgaaattgcaaaagaaactcaagctagagttttggagacaatactaaaacacggagatgttgaagaagctgtgagaatagtaaaagaagtaatacaaaagcttgccaattatgaaattccaccagagaagctcgcaatatatgagcagataacaagaccattacatgagtataaggcgataggtcctcacgtagctgttgcaaagaaactagctgctaaaggagttaaaataaagccaggaatggtaattggatacatagtacttagaggcgatggtccaattagcaatagggcaattctagctgaggaatacgatcccaaaaagcacaagtatgacgcagaatattacattgagaaccaggttcttccagcggtacttaggatattggagggatttggatacagaaaggaagacctcagataccaaaagacaagacaagtcggcctaacttcctggcttaacattaaaaaatcctga

SEQ ID NO: 24 - DNA, 2325 bp, Artificial
  24
atgattctggacaccgattacatcaccgaagatggcaagccagttatccgcattttcaaaaaagagaatggtgaattcaagatcgaatatgatcgtaccttcgagccgtacttctatgctctgctgaaagacgatagcgcgattgaggaggtcaagaaaatcaccgcggagcgtcacggtacggttgttaccgtgaaacgcgtggagaaagtccagaagaaatttctgggtcgcccggttgaagtgtggaagctgtactttacgcatccgcaagatgttccggcgattcgcgataagattcgtgagcacccggcagtcattgacatctacgagtatgacattccgttcgccaagcgttatctgatcgataagggtctggtcccgatggagggtgacgaagaactgaagatgctggcgttcgacatcgaaactctgtaccacgagggtgaagagtttgccgagggtccgatcttgatgatttcctacgcggacgaagagggcgcacgtgttatcacgtggaaaaatgttgatctgccgtatgttgacgtcgtaagcaccgagcgtgagatgatcaaacgttttctgcgcgttgttaaagaaaaagatcctgacgtgctgatcacctacaacggtgacaatttcgatttcgcgtacctgaagaaacgttgcgaaaaactgggtattaacttcgcgctgggtcgcgatggctctgaaccgaagatccagcgcatgggtgatcgttttgcggtcgaggtgaagggtcgcattcatttcgacctgtacccggtgattcgtcgtaccatcaacttgccgacttacaccctggaagccgtctatgaagctgtatttggtcaaccgaaagaaaaagtgtacgctgaggaaattacgacggcgtgggaaaccggtgagaacctggagcgcgttgcacgttattctatggaggacgcgaaagttacctacgaactgggtaaagagttcctgccgatggaggcccaactgtcccgtctggtgggccaaagcctgtgggacgttagccgcagcagcaccggtaacttagttgaatggttcttgctgcgtaaggcatacgaacgcaatgagctggcgccgaacaaaccggacgagaaagaattggcgcgtcgccgccagagctatgagggtggttatgtcaaagaaccggagcgcggcttgtgggagaacatcgtctatttggattttcgtagcattgcaccgagcatcattatcacgcataatgtgagcccggatacgttgaatcgtgagggctgtaaggaatacgacgtggcgcctcaggttggccaccgtttctgcaaggactttccgggctttatcccgagcctgctgggtgatttgctggaggaacgtcagaaaatcaagaagaagatgaaagcaaccattgatccgatcgagcgcaaattactggactaccgtcaacgtgccatcaagatcctggcgaattcgtattatggttactatggctacgcgcgtgcgcgctggtattgcaaagagtgtgccgagagcgtgaccgcttggggtcgtgagtacattaccatgacgatcaaagagattgaagagaaatacggctttaaggttatctatagcgacaccgacggtttctttgcaactatccctggcgcagacgcagaaaccgttaagaaaaaggcaatggagtttctgaagtatatcaacgcgaagttgccaggcgccctggaactggagtacgagggcttctacaagcgtggctttttcgtgacgaaaaagaaatacgctgttattgatgaagagggcaagatcacgacccgtggcctggaaattgtgcgccgtgattggagcgaaattgcaaaagaaacgcaagcgcgtgtgctggaagcgctgctgaaggacggcgacgtcgaaaaagctgtgcgtattgttaaagaggtcaccgagaagctgagcaaatacgaggtcccgccagagaaattggtgattcacgaacagattacgcgtgacctgaaagactataaggccaccggtccgcatgtcgcagtggcgaagcgcctggcggctcgcggtgtgaagatccgtccgggtaccgtcattagctatatcgtgctgaagggcagcggtcgtatcggcgaccgtgcgattccgttcgacgaatttgatccgaccaaacacaaatatgatgcggaatactatattgagaaccaagtgctgccagccgttgagcgtattctgcgcgccttcggttaccgcaaggaagatctgcgttaccagaaaactcgtcaggtcggtctgtccgcatggctgaaaccgaagggcacctga

SEQ ID NO: 25 - DNA, 20 bp, Artificial
  25
agagtttgatcmtggctcag

SEQ ID NO: 26 - DNA, 20 bp, Artificial
  26
cggttaccttgttacgactt

SEQ ID NO: 27 - DNA, 22 bp, Artificial
  27
ccagccaattcatgagtcggtg

SEQ ID NO: 28 - DNA, 22 bp, Artificial
  28
cctgacaactcgcaagtagcac

SEQ ID NO: 29 - DNA, 35 bp, Artificial
  29
cctctgtcgtttcctttctctgtttttgtccgtgg

SEQ ID NO: 30 - DNA, 36 bp, Artificial
  30
acatcgacataaaaaaatcccgtaaaaaaagccgca

SEQ ID NO: 31 - DNA, 32 bp, Artificial
  31
cgggaatacgacggttacccaccacaagcacg

SEQ ID NO: 32 - DNA, 30 bp, Artificial
  32
gccgcatccagactcaaatcaacgaccaga

SEQ ID NO: 33 - DNA, 22 bp, Artificial
  33
gctcaatggggtacttcagggt

SEQ ID NO: 34 - DNA, 22 bp, Artificial
  34
gtggacgttacgtaaaaggccc